European Patent Application EP 4 711 462 A1, published March 18, 2026. Title: クロストリジオイデス・ディフィシル菌に結合する抗体. Applicant: 国立大学法人　東京大学. Application WO, filed May 10, 2024. The sequence listing filed with the application follows.

SEQUENCE LISTING (34 sequences)

SEQ ID NO: 1 - protein, 479 aa, Mus musculus
MKFSWVIFFLMAVVTGVNSEVQLQQSLAELVRPGASVKLSCTASGFNIKNTYMHWVKQRPEQDLEWIGRIDPANGYTKYAPKFQGKATITADTSSNAAYLQLSSLTSEDTAIYYCGRGYSNFDYWGQGTTLTVSSESARNPTIYPLTLPRALSSDPVIIGCLIHDYFPSGTMNVTWGKSGKDITTVNFPPALASGGGYTMSSQLTLPAVECPEGESVKCSVQHDSNAVQELDVKCSGPPPPCPPCPPSCHPSLSLQRPALEDLLLGSDASLTCTLNGLRNPEGAVFTWEPSTGKDAVQKKAVQNSCGCYSVSSVLPGCAERWNSGASFKCTVTHPESDTLTGTIAKITVNTFPPQVHLLPPPSEELALNELVSLTCLVRAFNPKEVLVRWLHGNEELSPESYLVFEPLKEPGEGATTYLVTSVLRVSAELWKQGDQYSCMVGHEALPMNFTQKTIDRLSGKPTNVSVSVIMSEGDGICY

SEQ ID NO: 2 - protein, 236 aa, Mus musculus
MDMRTPAQFLGILLLWFPGFKCDIKMTQSPSSMYASLGERVTITCKASQDINSYLSWFQQKPGKSPKTLTYRANRLVDGVPSKFSGSGSGQDYSLTISSLEYEDMGIYYCLQYDEFPLTFGAGTKLELKRADAAPTVSIFPPSSEQLTSGGASVVCFLNNFYPKDINVKWKIDGSERQNGVLNSWTDQDSKDSTYSMSSTLTLTKDEYERHNSYTCEATHKTSTSPIVKSFNRNEC

SEQ ID NO: 3 - protein, 135 aa, Mus musculus
MKFSWVIFFLMAVVTGVNSEVQLQQSLAELVRPGASVKLSCTASGFNIKNTYMHWVKQRPEQDLEWIGRIDPANGYTKYAPKFQGKATITADTSSNAAYLQLSSLTSEDTAIYYCGRGYSNFDYWGQGTTLTVSS

SEQ ID NO: 4 - protein, 129 aa, Mus musculus
MDMRTPAQFLGILLLWFPGFKCDIKMTQSPSSMYASLGERVTITCKASQDINSYLSWFQQKPGKSPKTLTYRANRLVDGVPSKFSGSGSGQDYSLTISSLEYEDMGIYYCLQYDEFPLTFGAGTKLELK

SEQ ID NO: 5 - protein, 8 aa, Mus musculus
GFNIKNTY

SEQ ID NO: 6 - protein, 8 aa, Mus musculus
IDPANGYT

SEQ ID NO: 7 - protein, 9 aa, Mus musculus
GRGYSNFDY

SEQ ID NO: 8 - protein, 6 aa, Mus musculus
QDINSY

SEQ ID NO: 9 - skipped

SEQ ID NO: 10 - protein, 9 aa, Mus musculus
LQYDEFPLT

SEQ ID NO: 11 - DNA, 1440 bp, Mus musculus
  source 1..1440: mol_type = other DNA
atgaaattcagctgggtcatcttcttcctgatggcagtggttacaggggtcaattcagaggttcagctgcagcagtctctggcagagcttgtgaggccaggggcctcagtcaagttgtcctgcacagcttctggcttcaacatcaaaaacacctatatgcactgggtgaagcagaggcctgaacaggacctggagtggattggaaggattgatcctgcgaatggttatactaaatatgccccgaagttccagggcaaggccactataactgcagacacatcctccaacgcagcctacctgcagctcagcagcctgacatctgaggacactgccatctattactgtggtagaggctatagtaactttgactattggggccaaggcaccactctcacagtctcctcagagtctgcgagaaatcccaccatctacccactgacactcccacgagctctgtcaagtgacccagtgataatcggctgcctgattcacgattacttcccttccggcacgatgaatgtgacctggggaaagagtgggaaggatataaccaccgtaaacttcccacctgccctggcctctgggggagggtacaccatgagcagccagttgaccctgccagctgtcgagtgcccagaaggagaatccgtgaaatgttccgtgcaacatgactctaacgccgtccaagaattggatgtgaagtgctctggtcctcctcctccttgtcctccttgtcctccttcctgccatcccagcctgtcactgcagcggccagctcttgaggacctgctcctgggttcagatgccagcctcacatgtactctgaatggcctgagaaatcctgagggagctgtcttcacctgggagccctccactgggaaggatgcagtgcagaagaaagctgtgcagaattcctgcggctgctacagtgtgtccagcgtcctgcctggctgtgctgagcgctggaacagtggcgcatcattcaagtgcacagttacccatcctgagtctgacaccttaactggcacaattgccaaaatcacagtgaacaccttcccaccccaggtccacctgctaccgccgccgtcggaggagctggccctgaatgagctcgtgtccctgacatgcctggtgcgagctttcaaccctaaagaagtgctggtgcgatggctgcatggaaatgaggagctgtccccagaaagctacctagtgtttgagcccctaaaggagccaggcgagggagccaccacctacctggtgacaagcgtgttgcgtgtatcagctgaactctggaaacagggtgaccagtactcctgcatggtgggccacgaggccttgcccatgaacttcacccagaagaccatcgaccgtctgtcgggtaaacccaccaatgtcagcgtgtctgtgatcatgtcagagggagatggcatctgctactga

SEQ ID NO: 12 - DNA, 711 bp, Mus musculus
  source 1..711: mol_type = other DNA
atggacatgaggacccctgctcagtttcttggaatcttgttgctctggtttccaggtttcaaatgtgacatcaagatgacccagtctccatcttccatgtatgcatctctaggagagagagtcactatcacttgcaaggcgagtcaggacataaatagttatttaagctggttccagcagaaaccagggaaatctcctaagaccctgacctatcgtgcaaacagattggtagatggggtcccatcaaaattcagtggcagtggatctgggcaagattattctctcaccatcagcagcctggagtatgaagatatgggaatttattattgtctacagtatgatgagtttccgctcacgttcggtgctgggaccaagctggagctgaaacgggctgatgctgcaccaactgtatccatcttcccaccatccagtgagcagttaacatctggaggtgcctcagtcgtgtgcttcttgaacaacttctaccccaaagacatcaatgtcaagtggaagattgatggcagtgaacgacaaaatggcgtcctgaacagttggactgatcaggacagcaaagacagcacctacagcatgagcagcaccctcacgttgaccaaggacgagtatgaacgacataacagctatacctgtgaggccactcacaagacatcaacttcacccattgtcaagagcttcaacaggaatgagtgttga

SEQ ID NO: 13 - protein, 140 aa, Mus musculus
MGWSWIFLLFLSGTAGVLSEVQLQQSGPEVVEPGASVKIPCKASGYTFTDYNMDWVKQSHGKSLEWIGDINPNNGGTIYNQKFKGQATLTVDKSSSTAYMELRSLTSEDTAVYYCAKSGYYGSGRYFDVWGTGTTVTVSS

SEQ ID NO: 14 - protein, 127 aa, Mus musculus
MVSTPQFLVFLLFWIPASRGDILLTQSPVILSVSPGERVSFSCRASQSIGSSIHWYQQRTNGSPRLLIKYASESISGIPSRFSGSGSGTDFTLTINSVASEDIADYYCQQSKSWPWTFGGGTKLEIK

SEQ ID NO: 15 - protein, 8 aa, Mus musculus
GYTFTDYN

SEQ ID NO: 16 - protein, 8 aa, Mus musculus
INPNNGGT

SEQ ID NO: 17 - protein, 14 aa, Mus musculus
AKSGYYGSGRYFDV

SEQ ID NO: 18 - protein, 6 aa, Mus musculus
QSIGSS

SEQ ID NO: 19 - skipped

SEQ ID NO: 20 - protein, 9 aa, Mus musculus
QQSKSWPWT

SEQ ID NO: 21 - protein, 484 aa, Mus musculus
MGWSWIFLLFLSGTAGVLSEVQLQQSGPEVVEPGASVKIPCKASGYTFTDYNMDWVKQSHGKSLEWIGDINPNNGGTIYNQKFKGQATLTVDKSSSTAYMELRSLTSEDTAVYYCAKSGYYGSGRYFDVWGTGTTVTVSSESARNPTIYPLTLPRALSSDPVIIGCLIHDYFPSGTMNVTWGKSGKDITTVNFPPALASGGGYTMSSQLTLPAVECPEGESVKCSVQHDSNAVQELDVKCSGPPPPCPPCPPSCHPSLSLQRPALEDLLLGSDASLTCTLNGLRNPEGAVFTWEPSTGKDAVQKKAVQNSCGCYSVSSVLPGCAERWNSGASFKCTVTHPESDTLTGTIAKITVNTFPPQVHLLPPPSEELALNELVSLTCLVRAFNPKEVLVRWLHGNEELSPESYLVFEPLKEPGEGATTYLVTSVLRVSAELWKQGDQYSCMVGHEALPMNFTQKTIDRLSGKPTNVSVSVIMSEGDGICY

SEQ ID NO: 22 - protein, 234 aa, Mus musculus
MVSTPQFLVFLLFWIPASRGDILLTQSPVILSVSPGERVSFSCRASQSIGSSIHWYQQRTNGSPRLLIKYASESISGIPSRFSGSGSGTDFTLTINSVASEDIADYYCQQSKSWPWTFGGGTKLEIKRADAAPTVSIFPPSSEQLTSGGASVVCFLNNFYPKDINVKWKIDGSERQNGVLNSWTDQDSKDSTYSMSSTLTLTKDEYERHNSYTCEATHKTSTSPIVKSFNRNEC

SEQ ID NO: 23 - DNA, 1455 bp, Mus musculus
  source 1..1455: mol_type = other DNA
atgggatggagctggatctttctcctcttcctgtcaggaactgcaggtgtcctctctgaggtccaactgcaacagtctggacctgaagtggtggagcctggggcttcagtgaagataccctgcaaggcttctggatacacattcactgactacaacatggactgggtgaaacagagccatggaaagagccttgagtggattggcgatattaatccgaacaatggtggtactatctacaaccagaagttcaagggccaggccacattgactgttgacaagtcctccagtacagcctacatggagctccgcagcctgacatctgaggacactgcagtctattactgtgcaaaatcgggctactacggtagtggccggtacttcgatgtctggggcacagggaccacggtcaccgtctcctcagagtctgcgagaaatcccaccatctacccactgacactcccacgagctctgtcaagtgacccagtgataatcggctgcctgattcacgattacttcccttccggcacgatgaatgtgacctggggaaagagtgggaaggatataaccaccgtaaacttcccacctgccctggcctctgggggagggtacaccatgagcagccagttgaccctgccagctgtcgagtgcccagaaggagaatccgtgaaatgttccgtgcaacatgactctaacgccgtccaagaattggatgtgaagtgctctggtcctcctcctccttgtcctccttgtcctccttcctgccatcccagcctgtcactgcagcggccagctcttgaggacctgctcctgggttcagatgccagcctcacatgtactctgaatggcctgagaaatcctgagggagctgtcttcacctgggagccctccactgggaaggatgcagtgcagaagaaagctgtgcagaattcctgcggctgctacagtgtgtccagcgtcctgcctggctgtgctgagcgctggaacagtggcgcatcattcaagtgcacagttacccatcctgagtctgacaccttaactggcacaattgccaaaatcacagtgaacaccttcccaccccaggtccacctgctaccgccgccgtcggaggagctggccctgaatgagctcgtgtccctgacatgcctggtgcgagctttcaaccctaaagaagtgctggtgcgatggctgcatggaaatgaggagctgtccccagaaagctacctagtgtttgagcccctaaaggagccaggcgagggagccaccacctacctggtgacaagcgtgttgcgtgtatcagctgaactctggaaacagggtgaccagtactcctgcatggtgggccacgaggccttgcccatgaacttcacccagaagaccatcgaccgtctgtcgggtaaacccaccaatgtcagcgtgtctgtgatcatgtcagagggagatggcatctgctactga

SEQ ID NO: 24 - DNA, 705 bp, Mus musculus
  source 1..705: mol_type = other DNA
atggtatccacacctcagttccttgtatttttgcttttctggattccagcctccagaggtgacatcttgctgactcagtctccagtcatcctgtctgtgagtccaggagaaagagtcagtttctcctgcagggccagtcagagcattggctcaagcatacactggtatcagcaaagaacaaatggttctccaaggcttctcataaaatatgcttctgagtctatttctgggatcccttccaggtttagtggcagtggatcagggacagattttactcttaccatcaacagtgtggcgtctgaagacattgcagattattactgtcaacaaagtaaaagctggccgtggacgttcggtggaggcaccaaactggaaatcaaacgggctgatgctgcaccaactgtatccatcttcccaccatccagtgagcagttaacatctggaggtgcctcagtcgtgtgcttcttgaacaacttctaccccaaagacatcaatgtcaagtggaagattgatggcagtgaacgacaaaatggcgtcctgaacagttggactgatcaggacagcaaagacagcacctacagcatgagcagcaccctcacgttgaccaaggacgagtatgaacgacataacagctatacctgtgaggccactcacaagacatcaacttcacccattgtcaagagcttcaacaggaatgagtgttga

SEQ ID NO: 25 - DNA, 17 bp, synthetic construct
  source 1..17: mol_type = other DNA
  variation 1: note = S can be G or C
  variation 3: note = R can be A or G
  variation 6: note = N can be A, C, G or T
  variation 7: note = M can be A or C
  variation 13: note = S can be G or C
sargtnmagctgsagtc

SEQ ID NO: 26 - DNA, 23 bp, synthetic construct
  source 1..23: mol_type = other DNA
  variation 1: note = S can be G or C
  variation 3: note = R can be A or G
  variation 6: note = N can be A, C, G or T
  variation 7: note = M can be A or C
  variation 13: note = S can be G or C
  variation 16: note = S can be G or C
  variation 21: note = W can be A or T
sargtnmagctgsagsagtcwgg

SEQ ID NO: 27 - DNA, 21 bp, synthetic construct
  source 1..21: mol_type = other DNA
  variation 17: note = W can be A or T
  variation 19: note = S can be G or C
caggttactctgaaagwtstg

SEQ ID NO: 28 - DNA, 20 bp, synthetic construct
  source 1..20: mol_type = other DNA
  variation 9: note = R can be A or G
  variation 18: note = R can be A or G
gaggtccarctgcaacartc

SEQ ID NO: 29 - DNA, 20 bp, synthetic construct
  source 1..20: mol_type = other DNA
  variation 12: note = V can be G, C or A
  variation 18: note = R can be A or G
caggtccaactvcagcarcc

SEQ ID NO: 30 - DNA, 20 bp, synthetic construct
  source 1..20: mol_type = other DNA
  variation 9: note = S can be G or C
  variation 10: note = S can be G or C
gaggtgaasstggtggaatc

SEQ ID NO: 31 - DNA, 20 bp, synthetic construct
  source 1..20: mol_type = other DNA
gatgtgaacttggaagtgtc

SEQ ID NO: 32 - DNA, 22 bp, synthetic construct
  source 1..22: mol_type = other DNA
gatggtgggatttctcgcagac

SEQ ID NO: 33 - DNA, 32 bp, synthetic construct
  source 1..32: mol_type = other DNA
  variation 9: note = S can be G or C
  variation 24: note = R can be A or G
  variation 27: note = W can be A or T
  variation 30: note = R can be A or G
ggctgcagsttcagtggcagtggrtcwggrac

SEQ ID NO: 34 - DNA, 21 bp, synthetic construct
  source 1..21: mol_type = other DNA
aacgtgagggtgctgctcatg